European Patent Application EP 4 678 663 A1, published January 14, 2026. Title: NOVEL CORONAVIRUS PROTECTIVE NASAL SPRAY, AND PREPARATION AND USE THEREOF. Applicant: Sichuan Clover Biopharmaceuticals, Inc. Application EP 24766419.6, filed March 4, 2024. The sequence listing filed with the application follows.

SEQUENCE LISTING (18 sequences)

SEQ ID NO: 1 - protein, 978 aa, synthetic construct
MSSSSWLLLSLVAVTAAQSTIEEQAKTFLDKFNHEAEDLFYQSSLASWNYNTNITEENVQNMNNAGDKWSAFLKEQSTLAQMYPLQEIQNLTVKLQLQALQQNGSSVLSEDKSKRLNTILNTMSTIYSTGKVCNPDNPQECLLLEPGLNEIMANSLDYNERLWAWESWRSEVGKQLRPLYEEYVVLKNEMARANHYEDYGDYWRGDYEVNGVDGYDYSRGQLIEDVEHTFEEIKPLYEHLHAYVRAKLMNAYPSYISPIGCLPAHLLGDMWGRFWTNLYSLTVPFGQKPNIDVTDAMVDQAWDAQRIFKEAEKFFVSVGLPNMTQGFWENSMLTDPGNVQKAVCHPTAWDLGKGDFRILMCTKVTMDDFLTAHHEMGHIQYDMAYAAQPFLLRNGANEGFHEAVGEIMSLSAATPKHLKSIGLLSPDFQEDNETEINFLLKQALTIVGTLPFTYMLEKWRWMVFKGEIPKDQWMKKWWEMKREIVGVVEPVPHDETYCDPASLFHVSNDYSFIRYYTRTLYQFQFQEALCQAAKHEGPLHKCDISNSTEAGQKLFNMLRLGKSEPWTLALENVVGAKNMNVRPLLNYFEPLFTWLKDQNKNSFVGWSTDWSPYADQSIKVRISLKSALGDKAYEWNDNEMYLFRSSVAYAMRQYFLKVKNQMILFGEEDVRVANLKPRISFNFFVTAPKNVSDIIPRTEVEKAIRMSRSRINDAFRLNDNSLEFLGIQPTLGPPNQPPRSEPKSCDKTHTCPPCPAPELLGGPSVFLFPPKPKDTLMISRTPEVTCVVVDVSHEDPEVKFNWYVDGVEVHNAKTKPREEQYNSTYRVVSVLTVLHQDWLNGKEYKCKVSNKALPAPIEKTISKAKGQPREPQVYTLPPSRDELTKNQVSLTCLVKGFYPSDIAVEWESNGQPENNYKTTPPVLDSDGSFFLYSKLTVDKSRWQQGNVFSCSVMHEALHNHYTQKSLSLSPGKDSNLWN

SEQ ID NO: 2 - protein, 955 aa, synthetic construct
QSTIEEQAKTFLDKFNHEAEDLFYQSSLASWNYNTNITEENVQNMNNAGDKWSAFLKEQSTLAQMYPLQEIQNLTVKLQLQALQQNGSSVLSEDKSKRLNTILNTMSTIYSTGKVCNPDNPQECLLLEPGLNEIMANSLDYNERLWAWESWRSEVGKQLRPLYEEYVVLKNEMARANHYEDYGDYWRGDYEVNGVDGYDYSRGQLIEDVEHTFEEIKPLYEHLHAYVRAKLMNAYPSYISPIGCLPAHLLGDMWGRFWTNLYSLTVPFGQKPNIDVTDAMVDQAWDAQRIFKEAEKFFVSVGLPNMTQGFWENSMLTDPGNVQKAVCHPTAWDLGKGDFRILMCTKVTMDDFLTAHHEMGHIQYDMAYAAQPFLLRNGANEGFHEAVGEIMSLSAATPKHLKSIGLLSPDFQEDNETEINFLLKQALTIVGTLPFTYMLEKWRWMVFKGEIPKDQWMKKWWEMKREIVGVVEPVPHDETYCDPASLFHVSNDYSFIRYYTRTLYQFQFQEALCQAAKHEGPLHKCDISNSTEAGQKLFNMLRLGKSEPWTLALENVVGAKNMNVRPLLNYFEPLFTWLKDQNKNSFVGWSTDWSPYADQSIKVRISLKSALGDKAYEWNDNEMYLFRSSVAYAMRQYFLKVKNQMILFGEEDVRVANLKPRISFNFFVTAPKNVSDIIPRTEVEKAIRMSRSRINDAFRLNDNSLEFLGIQPTLGPPNQPPRSEPKSCDKTHTCPPCPAPELLGGPSVFLFPPKPKDTLMISRTPEVTCVVVDVSHEDPEVKFNWYVDGVEVHNAKTKPREEQYNSTYRVVSVLTVLHQDWLNGKEYKCKVSNKALPAPIEKTISKAKGQPREPQVYTLPPSRDELTKNQVSLTCLVKGFYPSDIAVEWESNGQPENNYKTTPPVLDSDGSFFLYSKLTVDKSRWQQGNVFSCSVMHEALHNHYTQKSLSLSPGK

SEQ ID NO: 3 - protein, 972 aa, synthetic construct
MSSSSWLLLSLVAVTAAQSTIEEQAKTFLDKFNHEAEDLFYQSSLASWNYNTNITEENVQNMNNAGDKWSAFLKEQSTLAQMYPLQEIQNLTVKLQLQALQQNGSSVLSEDKSKRLNTILNTMSTIYSTGKVCNPDNPQECLLLEPGLNEIMANSLDYNERLWAWESWRSEVGKQLRPLYEEYVVLKNEMARANHYEDYGDYWRGDYEVNGVDGYDYSRGQLIEDVEHTFEEIKPLYEHLHAYVRAKLMNAYPSYISPIGCLPAHLLGDMWGRFWTNLYSLTVPFGQKPNIDVTDAMVDQAWDAQRIFKEAEKFFVSVGLPNMTQGFWENSMLTDPGNVQKAVCHPTAWDLGKGDFRILMCTKVTMDDFLTAHHEMGHIQYDMAYAAQPFLLRNGANEGFHEAVGEIMSLSAATPKHLKSIGLLSPDFQEDNETEINFLLKQALTIVGTLPFTYMLEKWRWMVFKGEIPKDQWMKKWWEMKREIVGVVEPVPHDETYCDPASLFHVSNDYSFIRYYTRTLYQFQFQEALCQAAKHEGPLHKCDISNSTEAGQKLFNMLRLGKSEPWTLALENVVGAKNMNVRPLLNYFEPLFTWLKDQNKNSFVGWSTDWSPYADQSIKVRISLKSALGDKAYEWNDNEMYLFRSSVAYAMRQYFLKVKNQMILFGEEDVRVANLKPRISFNFFVTAPKNVSDIIPRTEVEKAIRMSRSRINDAFRLNDNSLEFLGIQPTLGPPNQPPRSEPKSCDKTHTCPPCPAPELLGGPSVFLFPPKPKDTLMISRTPEVTCVVVDVSHEDPEVKFNWYVDGVEVHNAKTKPREEQYNSTYRVVSVLTVLHQDWLNGKEYKCKVSNKALPAPIEKTISKAKGQPREPQVYTLPPSRDELTKNQVSLTCLVKGFYPSDIAVEWESNGQPENNYKTTPPVLDSDGSFFLYSKLTVDKSRWQQGNVFSCSVMHEALHNHYTQKSLSLSPGK

SEQ ID NO: 4 - protein, 961 aa, synthetic construct
QSTIEEQAKTFLDKFNHEAEDLFYQSSLASWNYNTNITEENVQNMNNAGDKWSAFLKEQSTLAQMYPLQEIQNLTVKLQLQALQQNGSSVLSEDKSKRLNTILNTMSTIYSTGKVCNPDNPQECLLLEPGLNEIMANSLDYNERLWAWESWRSEVGKQLRPLYEEYVVLKNEMARANHYEDYGDYWRGDYEVNGVDGYDYSRGQLIEDVEHTFEEIKPLYEHLHAYVRAKLMNAYPSYISPIGCLPAHLLGDMWGRFWTNLYSLTVPFGQKPNIDVTDAMVDQAWDAQRIFKEAEKFFVSVGLPNMTQGFWENSMLTDPGNVQKAVCHPTAWDLGKGDFRILMCTKVTMDDFLTAHHEMGHIQYDMAYAAQPFLLRNGANEGFHEAVGEIMSLSAATPKHLKSIGLLSPDFQEDNETEINFLLKQALTIVGTLPFTYMLEKWRWMVFKGEIPKDQWMKKWWEMKREIVGVVEPVPHDETYCDPASLFHVSNDYSFIRYYTRTLYQFQFQEALCQAAKHEGPLHKCDISNSTEAGQKLFNMLRLGKSEPWTLALENVVGAKNMNVRPLLNYFEPLFTWLKDQNKNSFVGWSTDWSPYADQSIKVRISLKSALGDKAYEWNDNEMYLFRSSVAYAMRQYFLKVKNQMILFGEEDVRVANLKPRISFNFFVTAPKNVSDIIPRTEVEKAIRMSRSRINDAFRLNDNSLEFLGIQPTLGPPNQPPRSEPKSCDKTHTCPPCPAPELLGGPSVFLFPPKPKDTLMISRTPEVTCVVVDVSHEDPEVKFNWYVDGVEVHNAKTKPREEQYNSTYRVVSVLTVLHQDWLNGKEYKCKVSNKALPAPIEKTISKAKGQPREPQVYTLPPSRDELTKNQVSLTCLVKGFYPSDIAVEWESNGQPENNYKTTPPVLDSDGSFFLYSKLTVDKSRWQQGNVFSCSVMHEALHNHYTQKSLSLSPGKDSNLWN

SEQ ID NO: 5 - protein, 721 aa, synthetic construct
QSTIEEQAKTFLDKFNHEAEDLFYQSSLASWNYNTNITEENVQNMNNAGDKWSAFLKEQSTLAQMYPLQEIQNLTVKLQLQALQQNGSSVLSEDKSKRLNTILNTMSTIYSTGKVCNPDNPQECLLLEPGLNEIMANSLDYNERLWAWESWRSEVGKQLRPLYEEYVVLKNEMARANHYEDYGDYWRGDYEVNGVDGYDYSRGQLIEDVEHTFEEIKPLYEHLHAYVRAKLMNAYPSYISPIGCLPAHLLGDMWGRFWTNLYSLTVPFGQKPNIDVTDAMVDQAWDAQRIFKEAEKFFVSVGLPNMTQGFWENSMLTDPGNVQKAVCHPTAWDLGKGDFRILMCTKVTMDDFLTAHHEMGHIQYDMAYAAQPFLLRNGANEGFHEAVGEIMSLSAATPKHLKSIGLLSPDFQEDNETEINFLLKQALTIVGTLPFTYMLEKWRWMVFKGEIPKDQWMKKWWEMKREIVGVVEPVPHDETYCDPASLFHVSNDYSFIRYYTRTLYQFQFQEALCQAAKHEGPLHKCDISNSTEAGQKLFNMLRLGKSEPWTLALENVVGAKNMNVRPLLNYFEPLFTWLKDQNKNSFVGWSTDWSPYADQSIKVRISLKSALGDKAYEWNDNEMYLFRSSVAYAMRQYFLKVKNQMILFGEEDVRVANLKPRISFNFFVTAPKNVSDIIPRTEVEKAIRMSRSRINDAFRLNDNSLEFLGIQPTLGPPNQPP

SEQ ID NO: 6 - protein, 232 aa, synthetic construct
EPKSCDKTHTCPPCPAPELLGGPSVFLFPPKPKDTLMISRTPEVTCVVVDVSHEDPEVKFNWYVDGVEVHNAKTKPREEQYNSTYRVVSVLTVLHQDWLNGKEYKCKVSNKALPAPIEKTISKAKGQPREPQVYTLPPSRDELTKNQVSLTCLVKGFYPSDIAVEWESNGQPENNYKTTPPVLDSDGSFFLYSKLTVDKSRWQQGNVFSCSVMHEALHNHYTQKSLSLSPGK

SEQ ID NO: 7 - protein, 738 aa, synthetic construct
MSSSSWLLLSLVAVTAAQSTIEEQAKTFLDKFNHEAEDLFYQSSLASWNYNTNITEENVQNMNNAGDKWSAFLKEQSTLAQMYPLQEIQNLTVKLQLQALQQNGSSVLSEDKSKRLNTILNTMSTIYSTGKVCNPDNPQECLLLEPGLNEIMANSLDYNERLWAWESWRSEVGKQLRPLYEEYVVLKNEMARANHYEDYGDYWRGDYEVNGVDGYDYSRGQLIEDVEHTFEEIKPLYEHLHAYVRAKLMNAYPSYISPIGCLPAHLLGDMWGRFWTNLYSLTVPFGQKPNIDVTDAMVDQAWDAQRIFKEAEKFFVSVGLPNMTQGFWENSMLTDPGNVQKAVCHPTAWDLGKGDFRILMCTKVTMDDFLTAHHEMGHIQYDMAYAAQPFLLRNGANEGFHEAVGEIMSLSAATPKHLKSIGLLSPDFQEDNETEINFLLKQALTIVGTLPFTYMLEKWRWMVFKGEIPKDQWMKKWWEMKREIVGVVEPVPHDETYCDPASLFHVSNDYSFIRYYTRTLYQFQFQEALCQAAKHEGPLHKCDISNSTEAGQKLFNMLRLGKSEPWTLALENVVGAKNMNVRPLLNYFEPLFTWLKDQNKNSFVGWSTDWSPYADQSIKVRISLKSALGDKAYEWNDNEMYLFRSSVAYAMRQYFLKVKNQMILFGEEDVRVANLKPRISFNFFVTAPKNVSDIIPRTEVEKAIRMSRSRINDAFRLNDNSLEFLGIQPTLGPPNQPP

SEQ ID NO: 8 - protein, 238 aa, synthetic construct
EPKSCDKTHTCPPCPAPELLGGPSVFLFPPKPKDTLMISRTPEVTCVVVDVSHEDPEVKFNWYVDGVEVHNAKTKPREEQYNSTYRVVSVLTVLHQDWLNGKEYKCKVSNKALPAPIEKTISKAKGQPREPQVYTLPPSRDELTKNQVSLTCLVKGFYPSDIAVEWESNGQPENNYKTTPPVLDSDGSFFLYSKLTVDKSRWQQGNVFSCSVMHEALHNHYTQKSLSLSPGKDSNLWN

SEQ ID NO: 9 - protein, 17 aa, synthetic construct
MSSSSWLLLSLVAVTAA

SEQ ID NO: 10 - protein, 6 aa, synthetic construct
DSNLWN

SEQ ID NO: 11 - protein, 740 aa, synthetic construct
MSSSSWLLLSLVAVTAAQSTIEEQAKTFLDKFNHEAEDLFYQSSLASWNYNTNITEENVQNMNNAGDKWSAFLKEQSTLAQMYPLQEIQNLTVKLQLQALQQNGSSVLSEDKSKRLNTILNTMSTIYSTGKVCNPDNPQECLLLEPGLNEIMANSLDYNERLWAWESWRSEVGKQLRPLYEEYVVLKNEMARANHYEDYGDYWRGDYEVNGVDGYDYSRGQLIEDVEHTFEEIKPLYEHLHAYVRAKLMNAYPSYISPIGCLPAHLLGDMWGRFWTNLYSLTVPFGQKPNIDVTDAMVDQAWDAQRIFKEAEKFFVSVGLPNMTQGFWENSMLTDPGNVQKAVCHPTAWDLGKGDFRILMCTKVTMDDFLTAHHEMGHIQYDMAYAAQPFLLRNGANEGFHEAVGEIMSLSAATPKHLKSIGLLSPDFQEDNETEINFLLKQALTIVGTLPFTYMLEKWRWMVFKGEIPKDQWMKKWWEMKREIVGVVEPVPHDETYCDPASLFHVSNDYSFIRYYTRTLYQFQFQEALCQAAKHEGPLHKCDISNSTEAGQKLFNMLRLGKSEPWTLALENVVGAKNMNVRPLLNYFEPLFTWLKDQNKNSFVGWSTDWSPYADQSIKVRISLKSALGDKAYEWNDNEMYLFRSSVAYAMRQYFLKVKNQMILFGEEDVRVANLKPRISFNFFVTAPKNVSDIIPRTEVEKAIRMSRSRINDAFRLNDNSLEFLGIQPTLGPPNQPPRS

SEQ ID NO: 12 - protein, 740 aa, synthetic construct
MSSSSWLLLSLVAVTAAQSTIEEQAKTFLDKFNHEAEDLFYQSSLASWNYNTNITEENVQNMNNAGDKWSAFLKEQSTLAQMYPLQEIQNLTVKLQLQALQQNGSSVLSEDKSKRLNTILNTMSTIYSTGKVCNPDNPQECLLLEPGLNEIMANSLDYNERLWAWESWRSEVGKQLRPLYEEYVVLKNEMARANHYEDYGDYWRGDYEVNGVDGYDYSRGQLIEDVEHTFEEIKPLYEHLHAYVRAKLMNAYPSYISPIGCLPAHLLGDMWGRFWTNLYSLTVPFGQKPNIDVTDAMVDQAWDAQRIFKEAEKFFVSVGLPNMTQGFWENSMLTDPGNVQKAVCHPTAWDLGKGDFRILMCTKVTMDDFLTAHHEMGHIQYDMAYAAQPFLLRNGANEGFHEAVGEIMSLSAATPKHLKSIGLLSPDFQEDNETEINFLLKQALTIVGTLPFTYMLEKWRWMVFKGEIPKDQWMKKWWEMKREIVGVVEPVPHDETYCDPASLFHVSNDYSFIRYYTRTLYQFQFQEALCQAAKHEGPLHKCDISNSTEAGQKLFNMLRLGKSEPWTLALENVVGAKNMNVRPLLNYFEPLFTWLKDQNKNSFVGWSTDWSPYADQSIKVRISLKSALGDKAYEWNDNEMYLFRSSVAYAMRQYFLKVKNQMILFGEEDVRVANLKPRISFNFFVTAPKNVSDIIPRTEVEKAIRMSRSRINDAFRLNDNSLEFLGIQPTLGPPNQPPVS

SEQ ID NO: 13 - protein, 723 aa, synthetic construct
QSTIEEQAKTFLDKFNHEAEDLFYQSSLASWNYNTNITEENVQNMNNAGDKWSAFLKEQSTLAQMYPLQEIQNLTVKLQLQALQQNGSSVLSEDKSKRLNTILNTMSTIYSTGKVCNPDNPQECLLLEPGLNEIMANSLDYNERLWAWESWRSEVGKQLRPLYEEYVVLKNEMARANHYEDYGDYWRGDYEVNGVDGYDYSRGQLIEDVEHTFEEIKPLYEHLHAYVRAKLMNAYPSYISPIGCLPAHLLGDMWGRFWTNLYSLTVPFGQKPNIDVTDAMVDQAWDAQRIFKEAEKFFVSVGLPNMTQGFWENSMLTDPGNVQKAVCHPTAWDLGKGDFRILMCTKVTMDDFLTAHHEMGHIQYDMAYAAQPFLLRNGANEGFHEAVGEIMSLSAATPKHLKSIGLLSPDFQEDNETEINFLLKQALTIVGTLPFTYMLEKWRWMVFKGEIPKDQWMKKWWEMKREIVGVVEPVPHDETYCDPASLFHVSNDYSFIRYYTRTLYQFQFQEALCQAAKHEGPLHKCDISNSTEAGQKLFNMLRLGKSEPWTLALENVVGAKNMNVRPLLNYFEPLFTWLKDQNKNSFVGWSTDWSPYADQSIKVRISLKSALGDKAYEWNDNEMYLFRSSVAYAMRQYFLKVKNQMILFGEEDVRVANLKPRISFNFFVTAPKNVSDIIPRTEVEKAIRMSRSRINDAFRLNDNSLEFLGIQPTLGPPNQPPRS

SEQ ID NO: 14 - protein, 723 aa, synthetic construct
QSTIEEQAKTFLDKFNHEAEDLFYQSSLASWNYNTNITEENVQNMNNAGDKWSAFLKEQSTLAQMYPLQEIQNLTVKLQLQALQQNGSSVLSEDKSKRLNTILNTMSTIYSTGKVCNPDNPQECLLLEPGLNEIMANSLDYNERLWAWESWRSEVGKQLRPLYEEYVVLKNEMARANHYEDYGDYWRGDYEVNGVDGYDYSRGQLIEDVEHTFEEIKPLYEHLHAYVRAKLMNAYPSYISPIGCLPAHLLGDMWGRFWTNLYSLTVPFGQKPNIDVTDAMVDQAWDAQRIFKEAEKFFVSVGLPNMTQGFWENSMLTDPGNVQKAVCHPTAWDLGKGDFRILMCTKVTMDDFLTAHHEMGHIQYDMAYAAQPFLLRNGANEGFHEAVGEIMSLSAATPKHLKSIGLLSPDFQEDNETEINFLLKQALTIVGTLPFTYMLEKWRWMVFKGEIPKDQWMKKWWEMKREIVGVVEPVPHDETYCDPASLFHVSNDYSFIRYYTRTLYQFQFQEALCQAAKHEGPLHKCDISNSTEAGQKLFNMLRLGKSEPWTLALENVVGAKNMNVRPLLNYFEPLFTWLKDQNKNSFVGWSTDWSPYADQSIKVRISLKSALGDKAYEWNDNEMYLFRSSVAYAMRQYFLKVKNQMILFGEEDVRVANLKPRISFNFFVTAPKNVSDIIPRTEVEKAIRMSRSRINDAFRLNDNSLEFLGIQPTLGPPNQPPVS

SEQ ID NO: 15 - protein, 978 aa, synthetic construct
MSSSSWLLLSLVAVTAAQSTIEEQAKTFLDKFNHEAEDLFYQSSLASWNYNTNITEENVQNMNNAGDKWSAFLKEQSTLAQMYPLQEIQNLTVKLQLQALQQNGSSVLSEDKSKRLNTILNTMSTIYSTGKVCNPDNPQECLLLEPGLNEIMANSLDYNERLWAWESWRSEVGKQLRPLYEEYVVLKNEMARANHYEDYGDYWRGDYEVNGVDGYDYSRGQLIEDVEHTFEEIKPLYEHLHAYVRAKLMNAYPSYISPIGCLPAHLLGDMWGRFWTNLYSLTVPFGQKPNIDVTDAMVDQAWDAQRIFKEAEKFFVSVGLPNMTQGFWENSMLTDPGNVQKAVCHPTAWDLGKGDFRILMCTKVTMDDFLTAHHEMGHIQYDMAYAAQPFLLRNGANEGFHEAVGEIMSLSAATPKHLKSIGLLSPDFQEDNETEINFLLKQALTIVGTLPFTYMLEKWRWMVFKGEIPKDQWMKKWWEMKREIVGVVEPVPHDETYCDPASLFHVSNDYSFIRYYTRTLYQFQFQEALCQAAKHEGPLHKCDISNSTEAGQKLFNMLRLGKSEPWTLALENVVGAKNMNVRPLLNYFEPLFTWLKDQNKNSFVGWSTDWSPYADQSIKVRISLKSALGDKAYEWNDNEMYLFRSSVAYAMRQYFLKVKNQMILFGEEDVRVANLKPRISFNFFVTAPKNVSDIIPRTEVEKAIRMSRSRINDAFRLNDNSLEFLGIQPTLGPPNQPPVSEPKSCDKTHTCPPCPAPELLGGPSVFLFPPKPKDTLMISRTPEVTCVVVDVSHEDPEVKFNWYVDGVEVHNAKTKPREEQYNSTYRVVSVLTVLHQDWLNGKEYKCKVSNKALPAPIEKTISKAKGQPREPQVYTLPPSRDELTKNQVSLTCLVKGFYPSDIAVEWESNGQPENNYKTTPPVLDSDGSFFLYSKLTVDKSRWQQGNVFSCSVMHEALHNHYTQKSLSLSPGKDSNLWN

SEQ ID NO: 16 - protein, 955 aa, synthetic construct
QSTIEEQAKTFLDKFNHEAEDLFYQSSLASWNYNTNITEENVQNMNNAGDKWSAFLKEQSTLAQMYPLQEIQNLTVKLQLQALQQNGSSVLSEDKSKRLNTILNTMSTIYSTGKVCNPDNPQECLLLEPGLNEIMANSLDYNERLWAWESWRSEVGKQLRPLYEEYVVLKNEMARANHYEDYGDYWRGDYEVNGVDGYDYSRGQLIEDVEHTFEEIKPLYEHLHAYVRAKLMNAYPSYISPIGCLPAHLLGDMWGRFWTNLYSLTVPFGQKPNIDVTDAMVDQAWDAQRIFKEAEKFFVSVGLPNMTQGFWENSMLTDPGNVQKAVCHPTAWDLGKGDFRILMCTKVTMDDFLTAHHEMGHIQYDMAYAAQPFLLRNGANEGFHEAVGEIMSLSAATPKHLKSIGLLSPDFQEDNETEINFLLKQALTIVGTLPFTYMLEKWRWMVFKGEIPKDQWMKKWWEMKREIVGVVEPVPHDETYCDPASLFHVSNDYSFIRYYTRTLYQFQFQEALCQAAKHEGPLHKCDISNSTEAGQKLFNMLRLGKSEPWTLALENVVGAKNMNVRPLLNYFEPLFTWLKDQNKNSFVGWSTDWSPYADQSIKVRISLKSALGDKAYEWNDNEMYLFRSSVAYAMRQYFLKVKNQMILFGEEDVRVANLKPRISFNFFVTAPKNVSDIIPRTEVEKAIRMSRSRINDAFRLNDNSLEFLGIQPTLGPPNQPPVSEPKSCDKTHTCPPCPAPELLGGPSVFLFPPKPKDTLMISRTPEVTCVVVDVSHEDPEVKFNWYVDGVEVHNAKTKPREEQYNSTYRVVSVLTVLHQDWLNGKEYKCKVSNKALPAPIEKTISKAKGQPREPQVYTLPPSRDELTKNQVSLTCLVKGFYPSDIAVEWESNGQPENNYKTTPPVLDSDGSFFLYSKLTVDKSRWQQGNVFSCSVMHEALHNHYTQKSLSLSPGK

SEQ ID NO: 17 - protein, 972 aa, synthetic construct
MSSSSWLLLSLVAVTAAQSTIEEQAKTFLDKFNHEAEDLFYQSSLASWNYNTNITEENVQNMNNAGDKWSAFLKEQSTLAQMYPLQEIQNLTVKLQLQALQQNGSSVLSEDKSKRLNTILNTMSTIYSTGKVCNPDNPQECLLLEPGLNEIMANSLDYNERLWAWESWRSEVGKQLRPLYEEYVVLKNEMARANHYEDYGDYWRGDYEVNGVDGYDYSRGQLIEDVEHTFEEIKPLYEHLHAYVRAKLMNAYPSYISPIGCLPAHLLGDMWGRFWTNLYSLTVPFGQKPNIDVTDAMVDQAWDAQRIFKEAEKFFVSVGLPNMTQGFWENSMLTDPGNVQKAVCHPTAWDLGKGDFRILMCTKVTMDDFLTAHHEMGHIQYDMAYAAQPFLLRNGANEGFHEAVGEIMSLSAATPKHLKSIGLLSPDFQEDNETEINFLLKQALTIVGTLPFTYMLEKWRWMVFKGEIPKDQWMKKWWEMKREIVGVVEPVPHDETYCDPASLFHVSNDYSFIRYYTRTLYQFQFQEALCQAAKHEGPLHKCDISNSTEAGQKLFNMLRLGKSEPWTLALENVVGAKNMNVRPLLNYFEPLFTWLKDQNKNSFVGWSTDWSPYADQSIKVRISLKSALGDKAYEWNDNEMYLFRSSVAYAMRQYFLKVKNQMILFGEEDVRVANLKPRISFNFFVTAPKNVSDIIPRTEVEKAIRMSRSRINDAFRLNDNSLEFLGIQPTLGPPNQPPVSEPKSCDKTHTCPPCPAPELLGGPSVFLFPPKPKDTLMISRTPEVTCVVVDVSHEDPEVKFNWYVDGVEVHNAKTKPREEQYNSTYRVVSVLTVLHQDWLNGKEYKCKVSNKALPAPIEKTISKAKGQPREPQVYTLPPSRDELTKNQVSLTCLVKGFYPSDIAVEWESNGQPENNYKTTPPVLDSDGSFFLYSKLTVDKSRWQQGNVFSCSVMHEALHNHYTQKSLSLSPGK

SEQ ID NO: 18 - protein, 961 aa, synthetic construct
QSTIEEQAKTFLDKFNHEAEDLFYQSSLASWNYNTNITEENVQNMNNAGDKWSAFLKEQSTLAQMYPLQEIQNLTVKLQLQALQQNGSSVLSEDKSKRLNTILNTMSTIYSTGKVCNPDNPQECLLLEPGLNEIMANSLDYNERLWAWESWRSEVGKQLRPLYEEYVVLKNEMARANHYEDYGDYWRGDYEVNGVDGYDYSRGQLIEDVEHTFEEIKPLYEHLHAYVRAKLMNAYPSYISPIGCLPAHLLGDMWGRFWTNLYSLTVPFGQKPNIDVTDAMVDQAWDAQRIFKEAEKFFVSVGLPNMTQGFWENSMLTDPGNVQKAVCHPTAWDLGKGDFRILMCTKVTMDDFLTAHHEMGHIQYDMAYAAQPFLLRNGANEGFHEAVGEIMSLSAATPKHLKSIGLLSPDFQEDNETEINFLLKQALTIVGTLPFTYMLEKWRWMVFKGEIPKDQWMKKWWEMKREIVGVVEPVPHDETYCDPASLFHVSNDYSFIRYYTRTLYQFQFQEALCQAAKHEGPLHKCDISNSTEAGQKLFNMLRLGKSEPWTLALENVVGAKNMNVRPLLNYFEPLFTWLKDQNKNSFVGWSTDWSPYADQSIKVRISLKSALGDKAYEWNDNEMYLFRSSVAYAMRQYFLKVKNQMILFGEEDVRVANLKPRISFNFFVTAPKNVSDIIPRTEVEKAIRMSRSRINDAFRLNDNSLEFLGIQPTLGPPNQPPVSEPKSCDKTHTCPPCPAPELLGGPSVFLFPPKPKDTLMISRTPEVTCVVVDVSHEDPEVKFNWYVDGVEVHNAKTKPREEQYNSTYRVVSVLTVLHQDWLNGKEYKCKVSNKALPAPIEKTISKAKGQPREPQVYTLPPSRDELTKNQVSLTCLVKGFYPSDIAVEWESNGQPENNYKTTPPVLDSDGSFFLYSKLTVDKSRWQQGNVFSCSVMHEALHNHYTQKSLSLSPGKDSNLWN